European Patent Application EP 4 141 121 A1, published March 1, 2023. Title: Recombinant hemagglutinin protein derived from influenza virus surface protein forming trimer and use thereof. Applicant: POSTECH ACADEMY-INDUSTRY FOUNDATION BioApplications Inc. INDUSTRY-ACADEMIC COOPERATION FOUNDATION GYEONGSANG NATIONAL UNIVERSITY KONKUK UNIVERSITY INDUSTRIAL COOPERATION CORP. The sequence listing filed with the application follows.

SEQUENCE LISTING (18 sequences)

SEQ ID NO: 1 - DNA, 1545 bp, Artificial
  H5N6 HA
gatcagatttgtattggatatcatgcgaacaactctacagagcaggttgatacaataatggaaaagaatgtgaccgttacacatgctcaagacatattggagaagacgcacaacgggaggctttgtgatctcaatggagttaaaccacttatacttaaggactgcagtgttgccggttggcttctgggaaacccaatgtgcgatgagtttattcgtgttcccgaatggagctacatcgtcgagagagctaacccagcaaatgatctgtgttatccagggaatctcaacgattacgaggaacttaagcatctactttcgagaatcaaccatttcgaaaagacacttattattcctaagtctagttggcctaatcacgaaacctcccttggtgtaagtgcagcatgcccttatcaaggtatgccgtcttttttccgaaacgtggtttggttgactaagaagaatgatgcttaccctactatcaagatgagctataataacaccaacagggaggaccttcttattttgtggggtattcaccattctaacaatgccgctgaacagactaatttgtacaagaaccctactacttatgtttcagtaggcacgtcaactttgaatcagagattggtcccaaaaatcgctacccgtagtcaagttaatggtcagagagggaggatggacttcttttggactattcttaagccaaatgatgctatacattttgagagcaatggaaactttatcgctcccgagtacgcctataagatagtaaagaagggcgattccactatcatgaagtctgaaatggaatatggtcattgcaatacgaagtgtcaaaccccgattggtgcaattaactcatctatgcctttccacaacattcacccactaactatcggagagtgtcctaaatacgtcaaatcaaataaattggtgcttgctacaggtctgcgcaactcccctttaagggagcgaagaagaaagaggggtttgtttggagctattgcaggcttcattgagggtggatggcaaggtatggtggatggctggtacggatatcatcattcgaatgaacaggggtctggttatgcagcggatcgggagagtacacaaaaggccatagatggagttaccaacaaggtaaactctattattgataaaatgaacacacagtttgaggctgtggggagggagttcaacaaccttgaaaggcgtatcgaaaacctcaacaaaaagatggaagacggctttctggacgtttggacttacaacgcagaattgctcgttcttatggaaaacgaacgtactttggatttccatgattctaacgtcaagaatctctacgataaagtgaggctgcaacttagggacaatgcaaaagaactaggtaacggttgctttgaattttatcacaagtgtgataatgagtgtatggagagtgtaagaaacgggacttatgactaccctcagtatagtgaggaagctagactcaagcgcgaggagatttccggagttaagcttgaatcaattggaacataccagatt

SEQ ID NO: 2 - protein, 515 aa, Artificial
  H5N6 HA
DQICIGYHANNSTEQVDTIMEKNVTVTHAQDILEKTHNGRLCDLNGVKPLILKDCSVAGWLLGNPMCDEFIRVPEWSYIVERANPANDLCYPGNLNDYEELKHLLSRINHFEKTLIIPKSSWPNHETSLGVSAACPYQGMPSFFRNVVWLTKKNDAYPTIKMSYNNTNREDLLILWGIHHSNNAAEQTNLYKNPTTYVSVGTSTLNQRLVPKIATRSQVNGQRGRMDFFWTILKPNDAIHFESNGNFIAPEYAYKIVKKGDSTIMKSEMEYGHCNTKCQTPIGAINSSMPFHNIHPLTIGECPKYVKSNKLVLATGLRNSPLRERRRKRGLFGAIAGFIEGGWQGMVDGWYGYHHSNEQGSGYAADRESTQKAIDGVTNKVNSIIDKMNTQFEAVGREFNNLERRIENLNKKMEDGFLDVWTYNAELLVLMENERTLDFHDSNVKNLYDKVRLQLRDNAKELGNGCFEFYHKCDNECMESVRNGTYDYPQYSEEARLKREEISGVKLESIGTYQI

SEQ ID NO: 3 - DNA, 96 bp, Artificial
  mCOr1
gtgtctaggcttgaggaagatgttagaaatctcaacgcaattgtccagaaacttcaggaaaggttggataggctggaggaaactgttcaagctaag

SEQ ID NO: 4 - protein, 32 aa, Artificial
  mCor1
VSRLEEDVRNLNAIVQKLQERLDRLEETVQAK

SEQ ID NO: 5 - DNA, 36 bp, Artificial
  Linker 1
ggaggttcaggaggttcaggaggttcaggaggttca

SEQ ID NO: 6 - protein, 12 aa, Artificial
  Linker 1
GGSGGSGGSGGS

SEQ ID NO: 7 - DNA, 18 bp, Artificial
  Linker 2
tcaggaggatcaggagga

SEQ ID NO: 8 - DNA, 6 bp, Artificial
  Linker 2
sggsgg

SEQ ID NO: 9 - DNA, 272 bp, Artificial
  BiP
atggctcgctcgtttggagctaacagtaccgttgtgttggcgatcatcttcttcggtgagtgattttccgatcttcttctccgatttagatctcctctacattgttgcttaatctcagaaccttttttcgttgttcctggatctgaatgtgtttgtttgcaatttcacgatcttaaaaggttagatctcgattggtattgacgattggaatctttacgatttcaggatgtttatttgcgttgtcctctgcaatagaagaggctacgaagtta

SEQ ID NO: 10 - DNA, 12 bp, Artificial
  HDEL
cacgatgagctc

SEQ ID NO: 11 - protein, 4 aa, Artificial
  HDEL
HDEL

SEQ ID NO: 12 - DNA, 21 bp, Artificial
  M17
ggcgtgtgtgtgtgttaaaga

SEQ ID NO: 13 - DNA, 303 bp, Artificial
  LysM
ggtaatactaactctgggggttcaacgaccaccattacaaacaacaacagtggaacaaattcatcttcaaccacctacaccgtgaagagtggcgatacgttgtggggaatcagtcaacgttatggtattagcgttgctcagatccagtctgcaaataaccttaagtctactataatttatattgggcaaaagctagttctgactggctcggctagtagcaccaattccggaggtagcaataactcagcttctactacccctacaacctctgtaactccagctaagcctacatcacagactaca

SEQ ID NO: 14 - protein, 101 aa, Artificial
  LysM
GNTNSGGSTTTITNNNSGTNSSSTTYTVKSGDTLWGISQRYGISVAQIQSANNLKSTIIYIGQKLVLTGSASSTNSGGSNNSASTTPTTSVTPAKPTSQTT

SEQ ID NO: 15 - DNA, 1220 bp, Artificial
  MacT
agagatctcctttgccccagagatcacaatggacgacttcctctatctctacgatctagtcaggaagttcgacggagaaggtgacgataccatgttcaccactgataatgagaagattagccttttcaatttcagaaagaatgctaacccacagatggttagagaggcttacgcagcaggtctcatcaagacgatctacccgagcaataatctccaggagatcaaataccttcccaagaaggttaaagatgcagtcaaaagattcaggactaactgcatcaagaacacagagaaagatatatttctcaagatcagaagtactattccagtatggacgattcaaggcttgcttcacaaaccaaggcaagtaatagagattggagtctctaaaaaggtagttcccactgaatcaaaggccatggagtcaaagattcaaatagaggacctaacagaactcgccgtaaagactggcgaacagttcatacagagtctcttacgactcaatgacaagaagaaaatcttcgtcaacatggtggagcacgacacgcttgtctactccaaaaatatcaaagatacagtctcagaagaccaaagggcaattgagacttttcaacaaagggtaatatccggaaacctcctcggattccattgcccagctatctgtcactttattgtgaagatagtggaaaaggaaggtggctcctacaaatgccatcattgcgataaaggaaaggccatcgttgaagatgcctctgccgacagtggtcccaaagatggacccccacccacgaggagcatcgtggaaaaagaagacgttccaaccacgtcttcaaagcaagtggattgatgtgacgcaagacgtgacgtaagtatctgagctagtttttatttttctactaatttggtcgtttatttcggcgtgtaggacatggcaaccgggcctgaatttcgcgggtattctgtttctattccaactttttcttgatccgcagccattaacgacttttgaatagatacgctgacacgccaagcctcgctagtcaaaagtgtaccaaacaacgctttacagcaagaacggaatgcgcgtgacgctcgcggtgacgccatttcgccttttcagaaatggataaatagccttgcttcctattatatcttcccaaattaccaatacattacactagcatctgaatttcataaccaatctcgatacaccaaatcgt

SEQ ID NO: 16 - DNA, 520 bp, Artificial
  RD29B terminator
aattttactcaaaatgttttggttgctatggtagggactatggggttttcggattccggtggaagtgagtggggaggcagtggcggaggtaagggagttcaagattctggaactgaagatttggggttttgcttttgaatgtttgcgtttttgtatgatgcctctgtttgtgaactttgatgtattttatctttgtgtgaaaaagagattgggttaataaaatatttgcttttttggataagaaactcttttagcggcccattaataaaggttacaaatgcaaaatcatgttagcgtcagatatttaattattcgaagatgattgtgatagatttaaaattatcctagtcaaaaagaaagagtaggttgagcagaaacagtgacatctgttgtttgtaccatacaaattagtttagattattggttaacatgttaaatggctatgcatgtgacatttagaccttatcggaattaatttgtagaattattaattaagatgttgattagttcaaacaaaaat

SEQ ID NO: 17 - DNA, 1518 bp, Artificial
  H9N2 HA
gataaaatttgcattggctaccagtcaacaaactccacagaaactgttgatacactagtagaaaacaatgtccctgtgacacataccaaagaattgctccacacagagcacaatggaatgttatgtgcaacaaacttgggacaccctcttatcctagacacctgcaccattgaagggttggtgtacggcaatccttcctgtgatttgctactgggagggaaagagtggtcttacattgtcgaaagatcatcagctgttaatgggatgtgctaccctggaagggtagagaatctggaagaactcaggtcctttttcagttctgctcgctcctacaaaagactcctactttttccagaccgtacttggaatgtgactttcaatgggacaagcaaagcatgctcaggctcattctacagaagtatgagatggctgacacacaagaacaattcttaccctattcaagacgcccaatataccaacgactggggaaagaatattctcttcatgtggggcatacaccatccacctactgatactgagcaaatgaatctatacaaaaaagctgatacaacaacaagtataacaacggaagatatcaatcgaactttcaaaccagggatagggccaaggcctcttgtcaatggtcaacaaggaagaattgattattattggtcagtactaaagccaggccagacattgcgaataagatccaatggaaatctaattgccccatggtatggacacattctttcaggagaaagccatggaagaatcctgaagaccgatttgaatagtggcaactgcataatacaatgccaaactgagaaaggtggtttgaacacgaccttgccattccaaaatgtcagcaaatatgcatttgggaactgtcccaaatatgttggagtgaagagtctcaaactggcagttggtctaaggaatgtgcctgctacatcaggtagagggcttttcggtgccatagctggattcatagaaggaggttggccaggactagttgcaggctggtacgggtttcagcactcaaatgatcaaggggttggaatagccgcagacaaagaatcaactcaagaagcagttgataaaataacatccaaagtaaataatataatcgacaaaatgaacaagcagtatgaaatcattgatcatgagttcagtgagattgaagccagactcaatatgatcaacaataagattgatgaccaaatacaggacatctgggcgtacaatgcagaattactagtactgcttgaaaaccagaaaacactcgatgatcatgatgcaaatgtgaacaatctgtataataaggtgaagagagcattgggttcaaatgcaatagaggatgggaagggatgcttcgagttgtatcacaaatgtgatgatcaatgcatggaaacaattagaaacgggacttatgacaggctaaagtataaagaagaatcaaaactagaaaggcagaaaatagaaggggtaaaactggagtctgaagaaacatacaagatt

SEQ ID NO: 18 - protein, 506 aa, Artificial
  H9N2 HA
DKICIGYQSTNSTETVDTLVENNVPVTHTKELLHTEHNGMLCATNLGHPLILDTCTIEGLVYGNPSCDLLLGGKEWSYIVERSSAVNGMCYPGRVENLEELRSFFSSARSYKRLLLFPDRTWNVTFNGTSKACSGSFYRSMRWLTHKNNSYPIQDAQYTNDWGKNILFMWGIHHPPTDTEQMNLYKKADTTTSITTEDINRTFKPGIGPRPLVNGQQGRIDYYWSVLKPGQTLRIRSNGNLIAPWYGHILSGESHGRILKTDLNSGNCIIQCQTEKGGLNTTLPFQNVSKYAFGNCPKYVGVKSLKLAVGLRNVPATSGRGLFGAIAGFIEGGWPGLVAGWYGFQHSNDQGVGIAADKESTQEAVDKITSKVNNIIDKMNKQYEIIDHEFSEIEARLNMINNKIDDQIQDIWAYNAELLVLLENQKTLDDHDANVNNLYNKVKRALGSNAIEDGKGCFELYHKCDDQCMETIRNGTYDRLKYKEESKLERQKIEGVKLESEETYKI